European Patent Specification EP 3 657 168 B1, published February 12, 2025. Title: TREATMENT OF AMYOTROPHIC LATERAL SCLEROSIS. Applicant: BRANDEIS UNIVERSITY. Application PCT/US2013/063858. The sequence listing filed with the application follows.

SEQUENCE LISTING (14 sequences)

SEQ ID NO: 1 - DNA, 3357 bp, Homo sapiens
atgagcgtggaggcgtacgggcccagctcgcagactctcactttcctggacacggaggaggccgagctgcttggcgccgacacacagggctccgagttcgagttcaccgactttactcttcctagccagacgcagacgccccccggcggccccggcggcccgggcggtggcggcgcgggaagcccgggcggcgcgggcgccggcgctgcggcgggacagctcgacgcgcaggttgggcccgaaggcatcctgcagaacggggctgtggacgacagtgtagccaagaccagccagttgttggctgagttgaacttcgaggaagatgaagaagacacctattacacgaaggacctccccatacacgcctgcagttactgtggaatacacgatcctgcctgcgtggtttactgtaataccagcaagaagtggttctgcaacggacgtggaaatacttctggcagccacattgtaaatcaccttgtgagggcaaaatgcaaagaggtgaccctgcacaaggacgggcccctgggggagacagtcctggagtgctacaactgcggctgtcgcaacgtcttcctcctcggcttcatcccggccaaagctgactcagtggtggtgctgctgtgcaggcagccctgtgccagccagagcagcctcaaggacatcaactgggacagctcgcagtggcagccgctgatccaggaccgctgcttcctgtcctggctggtcaagatcccctccgagcaggagcagctgcgggcacgccagatcacggcacagcagatcaacaagctggaggagctgtggaaggaaaacccttctgccacgctggaggacctggagaagccgggggtggacgaggagccgcagcatgtcctcctgcggtacgaggacgcctaccagtaccagaacatattcgggcccctggtcaagctggaggccgactacgacaagaagctgaaggagtcccagactcaagataacatcactgtcaggtgggacctgggccttaacaagaagagaatcgcctacttcactttgcccaagactgactctgacatgcggctcatgcagggggatgagatatgcctgcggtacaaaggggaccttgcgcccctgtggaaagggatcggccacgtcatcaaggtccctgataattatggcgatgagatcgccattgagctgcggagcagcgtgggtgcacctgtggaggtgactcacaacttccaggtggattttgtgtggaagtcgacctcctttgacaggatgcagagcgcattgaaaacgtttgccgtggatgagacctcggtgtctggctacatctaccacaagctgttgggccacgaggtggaggacgtaatcaccaagtgccagctgcccaagcgcttcacggcgcagggcctccccgacctcaaccactcccaggtttatgccgtgaagactgtgctgcaaagaccactgagcctgatccagggcccgccaggcacggggaagacggtgacgtcggccaccatcgtctaccacctggcccggcaaggcaacgggccggtgctggtgtgtgctccgagcaacatcgccgtggaccagctaacggagaagatccaccagacggggctaaaggtcgtgcgcctctgcgccaagagccgtgaggccatcgactccccggtgtcttttctggccctgcacaaccagatcaggaacatggacagcatgcctgagctgcagaagctgcagcagctgaaagacgagactggggagctgtcgtctgccgacgagaagcggtaccgggccttgaagcgcaccgcagagagagagctgctgatgaacgcagatgtcatctgctgcacatgtgtgggcgccggtgacccgaggctggccaagatgcagttccgctccattttaatcgacgaaagcacccaggccaccgagccggagtgcatggttcccgtggtcctcggggccaagcagctgatccttgtaggcgaccactgccagctgggcccagtggtgatgtgcaagaaggcggccaaggccgggctgtcacagtcgctcttcgagcgcctggtggtgctgggcatccggcccatccgcctgcaggtccagtaccggatgcaccctgcactcagcgccttcccatccaacatcttctacgagggctccctccagaatggtgtcactgcagcggatcgtgtgaagaagggatttgacttccagtggccccaacccgataaaccgatgttcttctacgtgacccagggccaagaggagattgccagctcgggcacctcctacctgaacaggaccgaggctgcgaacgtggagaagatcaccacgaagttgctgaaggcaggcgccaagccggaccagattggcatcatcacgccctacgagggccagcgctcctacctggtgcagtacatgcagttcagcggctccctgcacaccaagctctaccaggaagtggagatcgccagtgtggacgcctttcagggacgcgagaaggacttcatcatcctgtcctgtgtgcgggccaacgagcaccaaggcattggctttttaaatgaccccaggcgtctgaacgtggccctgaccagagcaaggtatggcgtcatcattgtgggcaacccgaaggcactatcaaagcagccgctctggaaccacctgctgaactactataaggagcagaaggtgctggtggaggggccgctcaacaacctgcgtgagagcctcatgcagttcagcaagccacggaagctggtcaacactatcaacccgggagcccgcttcatgaccacagccatgtatgatgcccgggaggccatcatcccaggctccgtctatgatcggagcagccagggccggccttccagcatgtacttccagacccatgaccagattggcatgatcagtgccggccctagccacgtggctgccatgaacattcccatccccttcaacctggtcatgccacccatgccaccgcctggctattttggacaagccaacgggcctgctgcagggcgaggcaccccgaaaggcaagactggtcgtgggggacgccagaagaaccgctttgggcttcctggacccagccagactaacctccccaacagccaagccagccaggatgtggcgtcacagcccttctctcagggcgccctgacgcagggctacatctccatgagccagccttcccagatgagccagcccggcctctcccagccggagctgtcccaggacagttaccttggtgacgagtttaaatcacaaatcgacgtggcgctctcacaggactccacgtaccagggagagcgggcttaccagcatggcggggtgacggggctgtcccagtattaa

SEQ ID NO: 2 - protein, 1118 aa, Homo sapiens [sequence omitted]

SEQ ID NO: 3 - DNA, 3819 bp, Homo sapiens
atgccagctgagcgtaaaaagccagcaagtatggaagaaaaagactctttaccaaacaacaaggaaaaagactgcagtgaaaggcggacagtgagcagcaaggagaggccaaaagacgatatcaagctcactgccaagaaggaggtcagcaaggcccctgaagacaagaagaagagactggaagatgataagagaaaaaaggaagacaaggaacgcaagaaaaaagacgaagaaaaggtgaaggcagaggaagaatcaaagaaaaaagaagaggaagaaaaaaagaaacatcaagaggaagagagaaagaagcaagaagagcaggccaaacgtcagcaagaagaagaagcagctgctcagatgaaagaaaaagaagaatccattcagcttcatcaggaagcttgggaacgacatcatttaagaaaggaacttcgtagcaaaaaccaaaatgctccggacagccgaccagaggaaaacttcttcagccgcctcgactcaagtttgaagaaaaatactgcttttgtcaagaaactaaaaactattacagaacaacagagagactccttgtcccatgattttaatggcctaaatttaagcaaatacattgcagaagctgtagcttccatcgtggaagcaaaactaaaaatctctgatgtgaactgtgctgtgcacctctgctctctctttcaccagcgttatgctgactttgccccatcacttcttcaggtctggaaaaaacattttgaagcaaggaaagaggagaaaacacctaacatcaccaagttaagaactgatttgcgttttattgcagaattgacaatagttgggattttcactgacaaggaaggtctttccttaatctatgaacagctaaaaaatattattaatgctgatcgggagtcccacactcatgtctctgtagtgattagtttctgtcgacattgtggagatgatattgctggacttgtaccaaggaaagtaaagagtgctgcagagaagtttaatttgagttttcctcctagtgagataattagtccagagaaacaacagcccttccagaatcttttaaaagagtactttacgtctttgaccaaacacctgaaaagggaccacagggagctccagaatactgagagacaaaacaggcgcattctacattctaaaggggagctcagtgaagatagacataaacagtatgaggaatttgctatgtcttaccagaagctgctggcaaattctcaatccttagcagaccttttggatgaaaatatgccagatcttcctcaagacaaacccacaccagaagaacatgggcctggaattgatatattcacacctggtaaacctggagaatatgacttggaaggtggtatatgggaagatgaagatgctcggaatttttatgagaacctcattgatttgaaggcttttgtcccagccatcttgtttaaagacaatgaaaaaagttgtcagaataaagagtccaacaaagatgataccaaagaggcaaaagaatctaaggagaataaggaggtatcaagtcccgatgatttggaacttgagttggagaatctagaaattaatgatgacaccttagaattagagggtggagatgaagctgaagatcttacaaagaaacttcttgatgaacaagaacaagaagatgaggaagccagcactggatctcatctcaagctcatagtagatgctttcctacagcagttacccaactgtgtcaaccgagatctgatagacaaggcagcaatggatttttgcatgaacatgaacacaaaagcaaacaggaagaagttggtacgggcactcttcatagttcctagacaaaggttggatttgctaccattttatgcaagattggttgctacattgcatccctgcatgtctgatgtagcagaggatctttgttccatgctgaggggggatttcagatttcatgtacggaaaaaggaccagatcaatattgaaacaaagaataaaactgttcgttttataggagaactaactaagtttaagatgttcaccaaaaatgacacactgcattgtttaaagatgcttctgtcagacttctctcatcaccatattgaaatggcatgcaccctgctggagacatgtggacggtttcttttcagatctccagaatctcacctgaggaccagtgtacttttggagcaaatgatgagaaagaagcaagcaatgcatcttgatgcgagatacgtcacaatggtagagaatgcatattactactgcaacccacctccagctgaaaaaaccgtgaaaaagaaacgtcctcctctccaggaatatgtccggaaacttttgtacaaagatctctctaaggttaccaccgagaaggttttgagacagatgcgaaagctgccctggcaggaccaagaagtgaaagactatgttatttgttgtatgataaacatctggaatgtgaaatataatagtattcattgtgtagccaacctcttagcaggactagtgctctaccaagaggatgttgggatccacgttgtggatggagtgttagaagatattcgattaggaatggaggttaatcaacctaaatttaatcagaggcgcatcagcagtgccaagttcttaggagaactttacaattaccgaatggtggaatcagctgttattttcagaactctgtattcttttacctcatttggtgttaatcctgatggctctccaagttccctggacccacctgagcatcttttcagaattagactcgtatgcactattctggacacatgtggccagtactttgacagaggttccagtaaacgaaaacttgattgtttccttgtatattttcagcgttatgtttggtggaagaaaagtttggaggtttggacaaaagaccatccatttcctattgatatagattacatgatcagtgatacactagaactgctaagaccaaagatcaaactctgtaattctctggaagaatccatcaggcaggtacaagacttggaacgagaattcttaataaaactaggcctagtaaatgacaaagactcaaaagattctatgacagaaggagaaaatcttgaagaggatgaagaagaagaagaaggtggggctgaaacagaagaacaatctggaaatgaaagtgaagtaaatgagccagaagaagaggagggttctgataatgatgatgatgagggagaagaagaggaggaagagaatacagattaccttacagattccaataaggaaaatgaaaccgatgaagagaatactgaggtaatgattaaaggcggtggacttaagcatgtaccttgtgtagaagatgaggacttcattcaagctctggataaaatgatgctagaaaatctacagcaacgaagtggtgaatctgttaaagtgcaccaactagatgtggccattcctttgcatctcaaaagccagctgaggaaagggcccccactgggaggtggggaaggagaggctgagtctgcagacacaatgccgtttgtcatgttaacaagaaaaggcaataaacagcagtttaagatccttaatgtacccatgtcctctcaacttgctgcaaatcactggaaccagcaacaggcagaacaagaagagaggatgagaatgaagaagctcacactagatatcaatgaacggcaagaacaagaagattatcaagaaatgttgcagtctcttgcacagcgcccagctccagcaaacaccaatcgtgagaggcggcctcgctaccaacatccgaagggagcacctaatgcagatctaatctttaagactggtgggaggagacgttga

SEQ ID NO: 4 - protein, 1272 aa, Homo sapiens
MPAERKKPASMEEKDSLPNNKEKDCSERRTVSSKERPKDDIKLTAKKEVSKAPEDKKKRLEDDKRKKEDKERKKKDEEKVKAEEESKKKEEEEKKKHQEEERKKQEEQAKRQQEEEAAAQMKEKEESIQLHQEAWERHHLRKELRSKNQNAPDSRPEENFFSRLDSSLKKNTAFVKKLKTITEQQRDSLSHDFNGLNLSKYIAEAVASIVEAKLKISDVNCAVHLCSLFHQRYADFAPSLLQVWKKHFEARKEEKTPNITKLRTDLRFIAELTIVGIFTDKEGLSLIYEQLKNIINADRESHTHVSVVISFCRHCGDDIAGLVPRKVKSAAEKFNLSFPPSEIISPEKQQPFQNLLKEYFTSLTKHLKRDHRELQNTERQNRRILHSKGELSEDRHKQYEEFAMSYQKLLANSQSLADLLDENMPDLPQDKPTPEEHGPGIDIFTPGKPGEYDLEGGIWEDEDARNFYENLIDLKAFVPAILFKDNEKSCQNKESNKDDTKEAKESKENKEVSSPDDLELELENLEINDDTLELEGGDEAEDLTKKLLDEQEQEDEEASTGSHLKLIVDAFLQQLPNCVNRDLIDKAAMDFCMNMNTKANRKKLVRALFIVPRQRLDLLPFYARLVATLHPCMSDVAEDLCSMLRGDFRFHVRKKDQINIETKNKTVRFIGELTKFKMFTKNDTLHCLKMLLSDFSHHHIEMACTLLETCGRFLFRSPESHLRTSVLLEQMMRKKQAMHLDARYVTMVENAYYYCNPPPAEKTVKKKRPPLQEYVRKLLYKDLSKVTTEKVLRQMRKLPWQDQEVKDYVICCMINIWNVKYNSIHCVANLLAGLVLYQEDVGIHVVDGVLEDIRLGMEVNQPKFNQRRISSAKFLGELYNYRMVESAVIFRTLYSFTSFGVNPDGSPSSLDPPEHLFRIRLVCTILDTCGQYFDRGSSKRKLDCFLVYFQRYVWWKKSLEVWTKDHPFPIDIDYMISDTLELLRPKIKLCNSLEESIRQVQDLEREFLIKLGLVNDKDSKDSMTEGENLEEDEEEEEGGAETEEQSGNESEVNEPEEEEGSDNDDDEGEEEEEENTDYLTDSNKENETDEENTEVMIKGGGLKHVPCVEDEDFIQALDKMMLENLQQRSGESVKVHQLDVAIPLHLKSQLRKGPPLGGGEGEAESADTMPFVMLTRKGNKQQFKILNVPMSSQLAANHWNQQQAEQEERMRMKKLTLDINERQEQEDYQEMLQSLAQRPAPANTNRERRPRYQHPKGAPNADLIFKTGGRRR

SEQ ID NO: 5 - DNA, 1359 bp, Homo sapiens
atgctgtcggccctagaagtgcagttccaccgcgactcgcagcagcaggaggctgagacgccgccaacttcgtcctccggttgcgggggcggtgcgggcaaacctcgcgaggagaagaggacggccctgagcaaggtggtcatccgccgcctgcctccgggcctcaccaaggagcagctggaggagcagctgcgcccgctgccagcacacgactacttcgagttcttcgccgccgacctgagtctttatcctcatctctactcaagagcatacattaattttaggaatcctgatgacatccttctttttagagatcgttttgatggatatatcttccttgacagcaaaggcctagaatatcctgcagtggtagagtttgctccattccagaagatagccaaaaagaagctgagaaaaaaagatgccaagactggaagcatcgaagatgatccagaatataagaagtttttagaaacctactgtgtggaggaagagaagaccagtgccaaccctgagactctgctgggggagatggaggcgaagacaagagagctcattgctagaagaaccacacctcttttggaatatattaaaaatagaaaattagaaaagcagagaattcgagaagagaagcgagaagaacggaggaggagagagttagaaaagaaacgtttgcgggaagaggaaaaaagaagaagaagagaagaagaaagatgcaaaaaaaaagagacagataaacagaagaaaattgcagagaaagaagtaaggattaagcttcttaagaaaccagaaaagggagaggaaccaaccacagagaaaccaaaagaaagaggagaggagattgatactggaggtggcaagcaggaatcctgtgcccccggtgcagtcgtaaaagccaggcccatggaaggctcgctggaggagccccaggagacgtcacacagcggcagtgataaagagcacagggatgtggagagatctcaagaacaagaatctgaagcacaaagataccatgtggatgacggcaggaggcacagagctcaccacgagcctgaacggctttccagaaggagtgaggatgagcagagatgggggaaaggacctggccaagacagagggaagaaggggagccaggacagcggggctccgggggaggccatggagagactgggaagagcgcaaaggtgtgacgacagtccagcacccagaaaagagcgactggcaaacaaggaccggccagccttgcagctgtatgatccaggagctcgcttccgagcgcgagagtgtggcggaaacaggaggatctgcaaggcagaaggttcggggactggtcctgagaagagggaagaggcagagtga

SEQ ID NO: 6 - protein, 452 aa, Homo sapiens [sequence omitted]

SEQ ID NO: 7 - DNA, 10986 bp, Homo sapiens
atgagccgcagagccccggggtctcggctgagcagcggcggcggcggcggcggcaccaagtatccgcggagctggaatgactggcaacccagaactgatagtgcatcagccgacccagataatttaaaatattcttcatccagagatagaggtggttcttcctcttatggactgcaaccttcaaattcagctgtggtgtctcggcaaaggcacgatgataccagagtccacgctgacatacagaatgacgaaaagggtggctacagtgtcaatggaggatctggggaaaatacttatggtcggaagtcgttggggcaagagctgagggttaacaatgtgaccagccctgagttcaccagtgttcagcatggcagtcgtgctttagccaccaaagacatgaggaaatcacaggagagatcgatgtcttattctgatgagtctcgactgtcgaatcttcttcggaggatcacccgggaagacgacagagaccgaagattggctactgtaaagcagttgaaagaatttattcagcaaccagaaaataagctggtactagttaaacaattggataatatcttggctgctgtacatgacgtgcttaatgaaagtagcaaattgcttcaggagttgagacaggagggagcttgctgtcttggccttctttgtgcttctctgagctatgaggctgagaagatcttcaagtggatttttagcaaatttagctcatctgcaaaagatgaagttaaactcctctacttatgtgccacctacaaagcactagagactgtaggagaaaagaaagccttttcatctgtaatgcagcttgtaatgaccagcctgcagtctattcttgaaaatgtggatacaccagaattgctttgtaaatgtgttaagtgcattcttttggtggctcgatgttaccctcatattttcagcactaattttagggatacagttgatatattagttggatggcatatagatcatactcagaaaccttcgctcacgcagcaggtatctgggtggttgcagagtttggagccattttgggtagctgatcttgcattttctactactcttcttggtcagtttctggaagacatggaagcatatgctgaggacctcagccatgtggcctctggggaatcagtggatgaagatgtccctcctccatcagtgtcattaccaaagctggctgcacttctccgggtatttagtactgtggtgaggagcattggggaacgcttcagcccaattcggggtcctccaattactgaggcatatgtaacagatgttctgtacagagtaatgagatgtgtgacggctgcaaaccaggtgtttttttctgaggctgtgttgacagctgctaatgagtgtgttggtgttttgctcggcagcttggatcctagcatgactatacattgtgacatggtcattacatatggattagaccaactggagaattgccagacttgtggtaccgattatatcatctcagtcttgaatttactcacgctgattgttgaacagataaatacgaaactgccatcatcatttgtagaaaaactgtttataccatcatctaaactactattcttgcgttatcataaagaaaaagaggttgttgctgtagcccatgctgtttatcaagcagtgctcagcttgaagaatattcctgttttggagactgcctataagttaatattgggagaaatgacttgtgccctaaacaacctcctacacagtctacaacttcctgaggcctgttctgaaataaaacatgaggcttttaagaatcatgtgttcaatgtagacaatgcaaaatttgtagttatatttgacctcagtgccctgactacaattggaaatgccaaaaactcactaatagggatgtgggcgctatctccaactgtctttgcacttctgagtaagaatctgatgattgtgcacagtgacctggctgttcacttccctgccattcagtatgctgtgctctacacattgtattctcattgtaccaggcatgatcactttatctctagtagcctcagttcttcctctccttctttgtttgatggagctgtgattagcactgtaactacggctacaaagaaacatttctcaattatattaaatcttctgggaatattacttaagaaagataaccttaaccaggacacgaggaaactgttaatgacttgggctttggaagcagctgttttaatgaagaagtctgaaacatacgcacctttattctctcttccgtctttccataaattttgcaaaggccttttagccaacactctcgttgaagatgtgaatatctgtctgcaggcatgcagcagtctacatgctctgtcctcttccttgccagatgatcttttacagagatgtgtcgatgtttgccgtgttcaactagtgcacagtggaactcgtattcgacaagcatttggaaaactgttgaaatcaattcctttagatgttgtcctaagcaataacaatcacacagaaattcaagaaatttctttagcattaagaagtcacatgagtaaagcaccaagtaatacattccacccccaagatttctctgatgttattagttttattttgtatgggaactctcatagaacagggaaggacaattggttggaaagactgttctatagctgccagagactggataagcgtgaccagtcaacaattccacgcaatctcctgaagacagatgctgtcctttggcagtgggccatatgggaagctgcacaattcactgttctttctaagctgagaaccccactgggcagagctcaagacaccttccagacaattgaaggtatcattcgaagtctcgcagctcacacattaaaccctgatcaggatgttagtcagtggacaactgcagacaatgatgaaggccatggtaacaaccaacttagacttgttcttcttctgcagtatctggaaaatctggagaaattaatgtataatgcatacgagggatgtgctaatgcattaacttcacctcccaaggtcattagaacttttttctataccaatcgccaaacttgtcaggactggctaacgcggattcgactctccatcatgagggtaggattgttggcaggccagcctgcagtgacagtgagacatggctttgacttgcttacagagatgaaaacaaccagcctatctcaggggaatgaattggaagtaaccattatgatggtggtagaagcattatgtgaacttcattgtcctgaagctatacagggaattgctgtctggtcatcatctattgttggaaaaaatcttctgtggattaactcagtggctcaacaggctgaagggaggtttgaaaaggcctctgtggagtaccaggaacacctgtgtgccatgacaggtgttgattgctgcatctccagctttgacaaatcggtgctcaccttagccaatgctgggcgtaacagtgccagcccgaaacattctctgaatggtgaatccagaaaaactgtgctgtccaaaccgactgactcttcccctgaggttataaattatttaggaaataaagcatgtgagtgctacatctcaattgccgattgggctgctgtgcaggaatggcagaacgctatccatgacttgaaaaagagtaccagtagcacttccctcaacctgaaagctgacttcaactatataaaatcattaagcagctttgagtctggaaaatttgttgaatgtaccgagcagttagaattgttaccaggagaaaatatcaatctacttgctggaggatcaaaagaaaaaatagacatgaaaaaactgcttcctaacatgttaagtccggatccgagggaacttcagaaatccattgaagttcaattgttaagaagttctgtttgtttggcaactgctttaaacccgatagaacaagatcagaagtggcagtctataactgaaaatgtggtaaagtacttgaagcaaacatcccgcatcgctattggacctctgagactttctactttaacagtttcacagtctttgccagttctaagtaccttgcagctgtattgctcatctgctttggagaacacagtttctaacagactttcaacagaggactgtcttattccactcttcagtgaagctttacgttcatgtaaacagcatgacgtgaggccatggatgcaggcattaaggtatactatgtaccagaatcagttgttggagaaaattaaagaacaaacagtcccaattagaagccatctcatggaattaggtctaacagcagcaaaatttgctagaaaacgagggaatgtgtcccttgcaacaagactgctggcacagtgcagtgaagttcagctgggaaagaccaccactgcacaggatttagtccaacattttaaaaaactatcaacccaaggtcaagtggatgaaaaatgggggcccgaacttgatattgaaaaaaccaaattgctttatacagcaggccagtcaacacatgcaatggaaatgttgagttcttgtgccatatctttctgcaagtctgtgaaagctgaatatgcagttgctaaatcaattctgacactggctaaatggatccaggcagaatggaaagagatttcaggacagctgaaacaggtttacagagctcagcaccaacagaacttcacaggtctttctactttgtctaaaaacatactcactctaatagaactgccatctgttaatacgatggaagaagagtatcctcggatcgagagtgaatctacagtgcatattggagttggagaacctgacttcattttgggacagttgtatcacctgtcttcagtacaggcacctgaagtagccaaatcttgggcagcgttggccagctgggcttataggtggggcagaaaggtggttgacaatgccagtcagggagaaggtgttcgtctgctgcctagagaaaaatctgaagttcagaatctacttccagacactataactgaggaagagaaagagagaatatatggtattcttggacaggctgtgtgtcggccggcggggattcaggatgaagatataacacttcagataactgagagtgaagacaacgaagaagatgacatggttgatgttatctggcgtcagttgatatcaagctgcccatggctttcagaacttgatgaaagtgcaactgaaggagttattaaagtgtggaggaaagttgtagatagaatattcagcctgtacaaactctcttgcagtgcatactttactttccttaaactcaacgctggtcaaattcctttagatgaggatgaccctaggctgcatttaagtcacagagtggaacagagcactgatgacatgattgtgatggccacattgcgcctgctgcggttgctcgtgaagcatgctggtgagcttcggcagtatctggagcacggcttggagacaacacccactgcaccatggagaggaattattccgcaacttttctcacgcttaaaccaccctgaagtgtatgtgcgccaaagtatttgtaaccttctctgccgtgtggctcaagattccccacatctcatattgtatcctgcaatagtgggtaccatatcgcttagtagtgaatcccaggcttcaggaaataaattttccactgcaattccaactttacttggcaatattcaaggagaagaattgctggtttctgaatgtgagggaggaagtcctcctgcatctcaggatagcaataaggatgaacctaaaagtggattaaatgaagaccaagccatgatgcaggattgttacagcaaaattgtagataagctgtcctctgcaaaccccaccatggtattacaggttcagatgctcgtggctgaactgcgcagggtcactgtgctctgggatgagctctggctgggagttttgctgcaacaacacatgtatgtcctgagacgaattcagcagcttgaagatgaggtgaagagagtccagaacaacaacaccttacgcaaagaagagaaaattgcaatcatgagggagaagcacacagctttgatgaagcccatcgtatttgctttggagcatgtgaggagtatcacagcggctcctgcagaaacacctcatgaaaaatggtttcaggataactatggtgatgccattgaaaatgccctagaaaaactgaagactccattgaaccctgcaaagcctgggagcagctggattccatttaaagagataatgctaagtttgcaacagagagcacagaaacgtgcaagttacatcttgcgtcttgaagaaatcagtccatggttggctgccatgactaacactgaaattgctcttcctggggaagtctcagccagagacactgtcacaatccatagtgtgggcggaaccatcacaatcttaccgactaaaaccaagccaaagaaacttctctttcttggatcagatgggaagagctatccttatcttttcaaaggactggaggatttacatctggatgagagaataatgcagttcctatctattgtgaataccatgtttgctacaattaatcgccaagaaacaccccggttccatgctcgacactattctgtaacaccactaggaacaagatcaggactaatccagtgggtagatggagccacacccttatttggtctttacaaacgatggcaacaacgggaagctgccttacaagcacaaaaggcccaagattcctaccaaactcctcagaatcctggaattgtaccccgtcctagtgaactttattacagtaaaattggccctgctttgaaaacagttgggcttagcctggatgtgtcccgtcgggattggcctcttcatgtaatgaaggcagtattggaagagttaatggaggccacacccccgaatctccttgccaaagagctctggtcatcttgcacaacacctgatgaatggtggagagttacgcagtcttatgcaagatctactgcagtcatgtctatggttggatacataattggccttggagacagacatctggataatgttcttatagatatgacgactggagaagttgttcacatagattacaatgtttgctttgaaaaaggtaaaagccttagagttcctgagaaagtaccttttcgaatgacacaaaacattgaaacagcactgggtgtaactggagtagaaggtgtatttaggctttcatgtgagcaggttttacacattatgcggcgtggcagagagaccctgctgacgctgctggaggcctttgtgtacgaccctctggtggactggacagcaggaggcgaggctgggtttgctggtgctgtctatggtggaggtggccagcaggccgagagcaagcagagcaagagagagatggagcgagagatcacccgcagcctgttttcttctagagtagctgagattaaggtgaactggtttaagaatagagatgagatgctggttgtgcttcccaagttggacggtagcttagatgaatacctaagcttgcaagagcaactgacagatgtggaaaaactgcagggcaaactactggaggaaatagagtttctagaaggagctgaaggggtggatcatccttctcatactctgcaacacaggtattctgagcacacccaactacagactcagcaaagagctgttcaggaagcaatccaggtgaagctgaatgaatttgaacaatggataacacattatcaggctgcattcaataatttagaagcaacacagcttgcaagcttgcttcaagagataagcacacaaatggaccttggtcctccaagttacgtgccagcaacagcctttctgcagaatgctggtcaggcccacttgattagccagtgcgagcagctggagggggaggttggtgctctcctgcagcagaggcgctccgtgctccgtggctgtctggagcaactgcatcactatgcaaccgtggccctgcagtatccgaaggccatatttcagaaacatcgaattgaacagtggaagacctggatggaagagctcatctgtaacaccacagtagagcgttgtcaagagctctataggaaatatgaaatgcaatatgctccccagccacccccaacagtgtgtcagttcatcactgccactgaaatgaccctgcagcgatacgcagcagacatcaacagcagacttattagacaagtggaacgcttgaaacaggaagctgtcactgtgccagtttgtgaagatcagttgaaagaaattgaacgttgcattaaagttttccttcatgagaatggagaagaaggatctttgagtctagcaagtgttattatttctgccctttgtacccttacaaggcgtaacctgatgatggaaggtgcagcgtcaagtgctggagaacagctggttgatctgacttctcgggatggagcctggttcttggaggaactctgcagtatgagcggaaacgtcacctgcttggttcagttactgaagcagtgccacctggtgccacaggacttagatatcccgaaccccatggaagcgtctgagacagttcacttagccaatggagtgtatacctcacttcaggaattgaattcgaatttccggcaaatcatatttccagaagcacttcgatgtttaatgaaaggggaatacacgttagaaagtatgctgcatgaactggacggtcttattgagcagaccaccgatggcgttcccctgcagactctagtggaatctcttcaggcctacttaagaaacgcagctatgggactggaagaagaaacacatgctcattacatcgatgttgccagactactacatgctcagtacggtgaattaatccaaccgagaaatggttcagttgatgaaacacccaaaatgtcagctggccagatgcttttggtagcattcgatggcatgtttgctcaagttgaaactgctttcagcttattagttgaaaagttgaacaagatggaaattcccatagcttggcgaaagattgacatcataagggaagccaggagtactcaagttaatttttttgatgatgataatcaccggcaggtgctagaagagattttctttctaaaaagactacagactattaaggagttcttcaggctctgtggtaccttttctaaaacattgtcaggatcaagttcacttgaagatcagaatactgtgaatgggcctgtacagattgtcaatgtgaaaaccctttttagaaactcttgtttcagtgaagaccaaatggccaaacctatcaaggcattcacagctgactttgtgaggcagctcttgatagggctacccaaccaagccctcggactcacactgtgcagttttatcagtgctctgggtgtagacatcattgctcaagtagaggcaaaggactttggtgccgaaagcaaagtttctgttgatgatctctgtaagaaagcggtggaacataacatccagatagggaagttctctcagctggttatgaacagggcaactgtgttagcaagttcttacgacactgcctggaagaagcatgacttggtgcgaaggctagaaaccagtatttcttcttgtaagacaagcctgcagcgggttcagctgcatattgccatgtttcagtggcaacatgaagatctacttatcaatagaccacaagccatgtcagtcacacctcccccacggtctgctatcctaaccagcatgaaaaagaagctgcataccctgagccagattgaaacttctattgcaacagttcaggagaagctagctgcacttgaatcaagtattgaacagcgactcaagtgggcaggtggtgccaaccctgcattggcccctgtactacaagattttgaagcaacgatagctgaaagaagaaatcttgtccttaaagagagccaaagagcaagtcaggtcacatttctctgcagcaatatcattcattttgaaagtttacgaacaagaactgcagaagccttaaacctggatgcggcgttatttgaactaatcaagcgatgtcagcagatgtgttcgtttgcatcacagtttaacagttcagtgtctgagttagagcttcgtttattacagagagtggacactggtcttgaacatcctattggcagctctgaatggcttttgtcagcacacaaacagttgacccaggatatgtctactcagagggcaattcagacagagaaagagcagcagatagaaacggtctgtgaaacaattcagaatctggttgataatataaagactgtgctcactggtcataaccgacagcttggagatgtcaaacatctcttgaaagctatggctaaggatgaagaagctgctctggcagatggtgaagatgttccctatgagaacagtgttaggcagtttttgggtgaatataaatcatggcaagacaacattcaaacagttctatttacattagtccaggctatgggtcaggttcgaagtcaagaacacgttgaaatgctccaggaaatcactcccaccttgaaagaactgaaaacacaaagtcagagtatctataataatttagtgagttttgcatcacccttagtcaccgatgcaacaaatgaatgttcgagtccaacgtcatctgctacttatcagccatccttcgctgcagcagtccggagtaacactggccagaagactcagcctgatgtcatgtcacagaatgctagaaagctgatccagaaaaatcttgctacatcagctgatactccaccaagcaccgttccaggaactggcaagagtgttgcttgtagtcctaaaaaggcagtcagagaccctaaaactgggaaagcggtgcaagagagaaactcctatgcagtgagtgtgtggaagagagtgaaagccaagttagagggccgagatgttgatccgaataggaggatgtcagttgctgaacaggttgactatgtcattaaggaagcaactaatctagataacttggctcagctgtatgaaggttggacagcctgggtgtga

SEQ ID NO: 8 - protein, 3661 aa, Homo sapiens
MSRRAPGSRLSSGGGGGGTKYPRSWNDWQPRTDSASADPDNLKYSSSRDRGGSSSYGLQPSNSAVVSRQRHDDTRVHADIQNDEKGGYSVNGGSGENTYGRKSLGQELRVNNVTSPEFTSVQHGSRALATKDMRKSQERSMSYSDESRLSNLLRRITREDDRDRRLATVKQLKEFIQQPENKLVLVKQLDNILAAVHDVLNESSKLLQELRQEGACCLGLLCASLSYEAEKIFKWIFSKFSSSAKDEVKLLYLCATYKALETVGEKKAFSSVMQLVMTSLQSILENVDTPELLCKCVKCILLVARCYPHIFSTNFRDTVDILVGWHIDHTQKPSLTQQVSGWLQSLEPFWVADLAFSTTLLGQFLEDMEAYAEDLSHVASGESVDEDVPPPSVSLPKLAALLRVFSTVVRSIGERFSPIRGPPITEAYVTDVLYRVMRCVTAANQVFFSEAVLTAANECVGVLLGSLDPSMTIHCDMVITYGLDQLENCQTCGTDYIISVLNLLTLIVEQINTKLPSSFVEKLFIPSSKLLFLRYHKEKEVVAVAHAVYQAVLSLKNIPVLETAYKLILGEMTCALNNLLHSLQLPEACSEIKHEAFKNHVFNVDNAKFVVIFDLSALTTIGNAKNSLIGMWALSPTVFALLSKNLMIVHSDLAVHFPAIQYAVLYTLYSHCTRHDHFISSSLSSSSPSLFDGAVISTVTTATKKHFSIILNLLGILLKKDNLNQDTRKLLMTWALEAAVLMKKSETYAPLFSLPSFHKFCKGLLANTLVEDVNICLQACSSLHALSSSLPDDLLQRCVDVCRVQLVHSGTRIRQAFGKLLKSIPLDVVLSNNNHTEIQEISLALRSHMSKAPSNTFHPQDFSDVISFILYGNSHRTGKDNWLERLFYSCQRLDKRDQSTIPRNLLKTDAVLWQWAIWEAAQFTVLSKLRTPLGRAQDTFQTIEGIIRSLAAHTLNPDQDVSQWTTADNDEGHGNNQLRLVLLLQYLENLEKLMYNAYEGCANALTSPPKVIRTFFYTNRQTCQDWLTRIRLSIMRVGLLAGQPAVTVRHGFDLLTEMKTTSLSQGNELEVTIMMVVEALCELHCPEAIQGIAVWSSSIVGKNLLWINSVAQQAEGRFEKASVEYQEHLCAMTGVDCCISSFDKSVLTLANAGRNSASPKHSLNGESRKTVLSKPTDSSPEVINYLGNKACECYISIADWAAVQEWQNAIHDLKKSTSSTSLNLKADFNYIKSLSSFESGKFVECTEQLELLPGENINLLAGGSKEKIDMKKLLPNMLSPDPRELQKSIEVQLLRSSVCLATALNPIEQDQKWQSITENVVKYLKQTSRIAIGPLRLSTLTVSQSLPVLSTLQLYCSSALENTVSNRLSTEDCLIPLFSEALRSCKQHDVRPWMQALRYTMYQNQLLEKIKEQTVPIRSHLMELGLTAAKFARKRGNVSLATRLLAQCSEVQLGKTTTAQDLVQHFKKLSTQGQVDEKWGPELDIEKTKLLYTAGQSTHAMEMLSSCAISFCKSVKAEYAVAKSILTLAKWIQAEWKEISGQLKQVYRAQHQQNFTGLSTLSKNILTLIELPSVNTMEEEYPRIESESTVHIGVGEPDFILGQLYHLSSVQAPEVAKSWAALASWAYRWGRKVVDNASQGEGVRLLPREKSEVQNLLPDTITEEEKERIYGILGQAVCRPAGIQDEDITLQITESEDNEEDDMVDVIWRQLISSCPWLSELDESATEGVIKVWRKVVDRIFSLYKLSCSAYFTFLKLNAGQIPLDEDDPRLHLSHRVEQSTDDMIVMATLRLLRLLVKHAGELRQYLEHGLETTPTAPWRGIIPQLFSRLNHPEVYVRQSICNLLCRVAQDSPHLILYPAIVGTISLSSESQASGNKFSTAIPTLLGNIQGEELLVSECEGGSPPASQDSNKDEPKSGLNEDQAMMQDCYSKIVDKLSSANPTMVLQVQMLVAELRRVTVLWDELWLGVLLQQHMYVLRRIQQLEDEVKRVQNNNTLRKEEKIAIMREKHTALMKPIVFALEHVRSITAAPAETPHEKWFQDNYGDAIENALEKLKTPLNPAKPGSSWIPFKEIMLSLQQRAQKRASYILRLEEISPWLAAMTNTEIALPGEVSARDTVTIHSVGGTITILPTKTKPKKLLFLGSDGKSYPYLFKGLEDLHLDERIMQFLSIVNTMFATINRQETPRFHARHYSVTPLGTRSGLIQWVDGATPLFGLYKRWQQREAALQAQKAQDSYQTPQNPGIVPRPSELYYSKIGPALKTVGLSLDVSRRDWPLHVMKAVLEELMEATPPNLLAKELWSSCTTPDEWWRVTQSYARSTAVMSMVGYIIGLGDRHLDNVLIDMTTGEVVHIDYNVCFEKGKSLRVPEKVPFRMTQNIETALGVTGVEGVFRLSCEQVLHIMRRGRETLLTLLEAFVYDPLVDWTAGGEAGFAGAVYGGGGQQAESKQSKREMEREITRSLFSSRVAEIKVNWFKNRDEMLVVLPKLDGSLDEYLSLQEQLTDVEKLQGKLLEEIEFLEGAEGVDHPSHTLQHRYSEHTQLQTQQRAVQEAIQVKLNEFEQWITHYQAAFNNLEATQLASLLQEISTQMDLGPPSYVPATAFLQNAGQAHLISQCEQLEGEVGALLQQRRSVLRGCLEQLHHYATVALQYPKAIFQKHRIEQWKTWMEELICNTTVERCQELYRKYEMQYAPQPPPTVCQFITATEMTLQRYAADINSRLIRQVERLKQEAVTVPVCEDQLKEIERCIKVFLHENGEEGSLSLASVIISALCTLTRRNLMMEGAASSAGEQLVDLTSRDGAWFLEELCSMSGNVTCLVQLLKQCHLVPQDLDIPNPMEASETVHLANGVYTSLQELNSNFRQIIFPEALRCLMKGEYTLESMLHELDGLIEQTTDGVPLQTLVESLQAYLRNAAMGLEEETHAHYIDVARLLHAQYGELIQPRNGSVDETPKMSAGQMLLVAFDGMFAQVETAFSLLVEKLNKMEIPIAWRKIDIIREARSTQVNFFDDDNHRQVLEEIFFLKRLQTIKEFFRLCGTFSKTLSGSSSLEDQNTVNGPVQIVNVKTLFRNSCFSEDQMAKPIKAFTADFVRQLLIGLPNQALGLTLCSFISALGVDIIAQVEAKDFGAESKVSVDDLCKKAVEHNIQIGKFSQLVMNRATVLASSYDTAWKKHDLVRRLETSISSCKTSLQRVQLHIAMFQWQHEDLLINRPQAMSVTPPPRSAILTSMKKKLHTLSQIETSIATVQEKLAALESSIEQRLKWAGGANPALAPVLQDFEATIAERRNLVLKESQRASQVTFLCSNIIHFESLRTRTAEALNLDAALFELIKRCQQMCSFASQFNSSVSELELRLLQRVDTGLEHPIGSSEWLLSAHKQLTQDMSTQRAIQTEKEQQIETVCETIQNLVDNIKTVLTGHNRQLGDVKHLLKAMAKDEEAALADGEDVPYENSVRQFLGEYKSWQDNIQTVLFTLVQAMGQVRSQEHVEMLQEITPTLKELKTQSQSIYNNLVSFASPLVTDATNECSSPTSSATYQPSFAAAVRSNTGQKTQPDVMSQNARKLIQKNLATSADTPPSTVPGTGKSVACSPKKAVRDPKTGKAVQERNSYAVSVWKRVKAKLEGRDVDPNRRMSVAEQVDYVIKEATNLDNLAQLYEGWTAWV

SEQ ID NO: 9 - DNA, 3051 bp, Homo sapiens
atgagccaaggcccccccacaggggagagcagcgagcccgaagcaaaagtcctccacactaagcggctttaccgggctgtggtggaggctgtgcatcgacttgacctcatcctttgcaacaaaactgcttatcaagaagtattcaaaccagaaaacattagcctgaggaacaagctgcgtgagctctgcgtcaagcttatgttcctgcacccagtggactatgggagaaaggctgaggagctgctgtggagaaaggtatactatgaagttatccagcttatcaagactaacaaaaagcacatccacagccggagcactttggaatgtgcctacaggacgcacctggttgctggtattggcttctaccagcatctccttctctatatccagtcccactaccagctggaactgcagtgctgcatcgactggacccatgtcactgaccccctcataggatgcaagaagccagtgtctgcctcagggaaggagatggattgggcacagatggcatgtcaccgatgtctggtgtatctgggggatttgtcccgatatcagaatgaattagctggcgtagataccgagctgctagccgagagattttactaccaagccctgtcagtagctcctcagattggaatgcccttcaatcagctgggcaccctggcaggcagcaagtactataatgtggaagccatgtattgctacctgcgctgcatccagtcagaagtgtcctttgagggagcctatgggaacctcaagcggctgtatgacaaggcagccaaaatgtaccaccaactgaagaagtgtgagactcggaaactgtctcctggcaaaaagcgatgtaaagacattaaaaggttgctagtgaactttatgtatctgcaaagcctcctacagcccaaaagcagctccgtggactcagagctgacctcactttgccagtcagtcctggaggacttcaacctctgcctcttctacctgccctcctcacccaacctcagcctggccagtgaggatgaggaggagtatgagagtggatatgctttcctcccggaccttctcatctttcaaatggtcatcatctgccttatgtgtgtgcacagcttggagagagcaggatccaagcagtacagtgcagccattgccttcaccctggccctcttttcccacctcgtcaatcatgtcaacatacggctgcaggctgagctggaagagggcgagaatcccgtcccggcattccagagtgatggcacagatgaaccagagtccaaggaacctgtggagaaagaggaggagccagatcctgagcctcctcctgtaacaccccaagtgggtgagggcagaaagagccgtaagttctctcgcctctcctgtctccgccgtcgccgccacccacccaaagttggtgatgacagtgacctgagtgaaggctttgaatcggactcaagccatgactcagcccgggccagtgagggctcagacagtggctctgacaagagtcttgaaggtgggggaacggcctttgatgctgaaacagactcggaaatgaatagccaggagtcccgatcagacttggaagatatggaggaagaggaggggacacggtcaccaaccctggagccccctcggggcagatcagaggctcccgattccctcaatggcccactgggccccagtgaggctagcattgccagcaatctacaagccatgtccacccagatgttccagactaagcgctgcttccgactggcccccacctttagcaacctgctcctccagcccaccaccaaccctcatacctcggccagccacaggccttgcgtcaatggggatgtagacaagccttcagagccagcctctgaggagggctctgagtcggaggggagtgagtccagtggacgctcctgtcggaatgagcgcagcatccaggagaagcttcaggtcctgatggccgaaggtctgcttcctgctgtgaaagtcttcctggactggcttcggaccaaccccgacctcatcatcgtgtgtgcgcagagctctcaaagtctgtggaaccgcctgtctgtgttgctgaatctgttgcctgctgctggtgaactccaggagtctggcctggccttgtgtcctgaggtccaagatcttcttgaaggttgtgaactgcctgacctcccctctagccttctgctcccagaggacatggctcttcgtaacctgcccccgctccgagctgcccacagacgctttaactttgacacggatcggcccctgctcagcaccttagaggagtcagtggtgcgcatctgctgcatccgcagctttggtcatttcatcgcccgcctgcaaggcagcatcctgcagttcaacccagaggttggcatcttcgtcagcattgcccagtctgagcaggagagcctgctgcagcaggcccaggcacagttccgaatggcacaggaggaagctcgtcggaacaggctcatgagagacatggctcagctacgacttcagctcgaagtgtctcagctggagggcagcctgcagcagcccaaggcccagtcagccatgtctccctacctcgtccctgacacccaggccctctgccaccatctccctgtcatccgccaactggccaccagtggccgcttcattgtcatcatcccaaggacagtgatcgatggcctggatttgctgaagaaggaacacccaggggcccgggatgggattcggtacctggaggcagagtttaaaaaaggaaacaggtacattcgctgccagaaagaggtgggaaagagctttgagcggcataagctgaagaggcaggatgcagatgcctggactctctataagatcctagacagctgcaaacagctgactctggcccagggggcaggtgaggaggatccgagtggcatggtgaccatcatcacaggccttccactggacaaccccagcgtgctttcaggccccatgcaggcagccctgcaggccgctgcccacgccagtgtggacatcaagaatgttctggacttctacaagcagtggaaggaaattggttga

SEQ ID NO: 10 - protein, 1016 aa, Homo sapiens
MSQGPPTGESSEPEAKVLHTKRLYRAVVEAVHRLDLILCNKTAYQEVFKPENISLRNKLRELCVKLMFLHPVDYGRKAEELLWRKVYYEVIQLIKTNKKHIHSRSTLECAYRTHLVAGIGFYQHLLLYIQSHYQLELQCCIDWTHVTDPLIGCKKPVSASGKEMDWAQMACHRCLVYLGDLSRYQNELAGVDTELLAERFYYQALSVAPQIGMPFNQLGTLAGSKYYNVEAMYCYLRCIQSEVSFEGAYGNLKRLYDKAAKMYHQLKKCETRKLSPGKKRCKDIKRLLVNFMYLQSLLQPKSSSVDSELTSLCQSVLEDFNLCLFYLPSSPNLSLASEDEEEYESGYAFLPDLLIFQMVIICLMCVHSLERAGSKQYSAAIAFTLALFSHLVNHVNIRLQAELEEGENPVPAFQSDGTDEPESKEPVEKEEEPDPEPPPVTPQVGEGRKSRKFSRLSCLRRRRHPPKVGDDSDLSEGFESDSSHDSARASEGSDSGSDKSLEGGGTAFDAETDSEMNSQESRSDLEDMEEEEGTRSPTLEPPRGRSEAPDSLNGPLGPSEASIASNLQAMSTQMFQTKRCFRLAPTFSNLLLQPTTNPHTSASHRPCVNGDVDKPSEPASEEGSESEGSESSGRSCRNERSIQEKLQVLMAEGLLPAVKVFLDWLRTNPDLIIVCAQSSQSLWNRLSVLLNLLPAAGELQESGLALCPEVQDLLEGCELPDLPSSLLLPEDMALRNLPPLRAAHRRFNFDTDRPLLSTLEESVVRICCIRSFGHFIARLQGSILQFNPEVGIFVSIAQSEQESLLQQAQAQFRMAQEEARRNRLMRDMAQLRLQLEVSQLEGSLQQPKAQSAMSPYLVPDTQALCHHLPVIRQLATSGRFIVIIPRTVIDGLDLLKKEHPGARDGIRYLEAEFKKGNRYIRCQKEVGKSFERHKLKRQDADAWTLYKILDSCKQLTLAQGAGEEDPSGMVTIITGLPLDNPSVLSGPMQAALQAAAHASVDIKNVLDFYKQWKEIG

SEQ ID NO: 11 - DNA, 1536 bp, Homo sapiens
atggagacattccctgcagtggctgagaaggtcctcaaggagttccaggtgttactgcagcacagcccctctcccattggaagtacccgcatgctgcagcttatgaccatcaatatgtttgcagtacacaactcccagctgaaagactgcttctcggaggagtgccgctctgtgatccaggaacaagccgcagctctgggcttggccatgttttctctactggtccgccgctgcacctgcttacttaaggagtccgccaaagctcagctgtcctctcctgaggaccaggatgaccaagacgacatcaaggtgtcttcctttgtcccggacctgaaggagctgctccccagtgtcaaagtctggtcagattggatgctcggctacccggacacctggaatcctcctcccacatccctggatctgccctcgcatgttgctgtggatgtatggtcgacgctggctgatttctgtaacatactgactgcagtgaatcagtctgaggtgccactgtacaaggacccggatgatgacctcacccttcttatcctggaagaggatcggcttctctcgggctttgtccccttgctggctgcccctcaggacccctgctacgtggagaaaacctcggataaggttattgcagctgactgcaaaagggtcacagtgctgaagtattttctggaagccctttgtggacaagaagagcctctgctggcattcaagggtggaaagtatgtgtcagtggcacccgtcccagacaccatgggaaaggaaatgggaagccaagagggaacacgactggaagatgaggaggaggatgtggtgattgaagactttgaggaagattcagaggctgaaggcagcggaggcgaggatgacatcagggagcttcgggccaagaagctggctctggccaggaagatagctgagcagcagcgtcgccaggaaaagatccaggctgtcctggaggaccacagtcagatgaggcagatggagctcgaaatcagacctttgttcctcgtaccagacaccaacggcttcattgaccacctggccagtctggcgcggctgctggagagcaggaagtacatcctggtggtgcccctcatcgtgatcaatgagctggacggcctggccaaggggcaggagacagaccaccgggctgggggctacgcccgtgtggtacaagagaaggcccgcaagtccatcgagttcctcgagcagcgattcgagagtcgggactcttgcctgcgagccctgaccagccgtggcaatgaactcgaatccatcgccttccgcagtgaggacatcactggccagctgggtaacaacgatgatctcatcctgtcctgctgcctccactactgcaaagacaaggctaaggacttcatgcccgccagcaaagaggagccaatccggctactgcgggaggtggtgctgttgacggatgaccggaacctgcgtgtgaaggcgctcacaaggaatgttcctgtacgggacatcccagccttcctcacgtgggcccaggtgggctga

SEQ ID NO: 12 - protein, 511 aa, Homo sapiens
METFPAVAEKVLKEFQVLLQHSPSPIGSTRMLQLMTINMFAVHNSQLKDCFSEECRSVIQEQAAALGLAMFSLLVRRCTCLLKESAKAQLSSPEDQDDQDDIKVSSFVPDLKELLPSVKVWSDWMLGYPDTWNPPPTSLDLPSHVAVDVWSTLADFCNILTAVNQSEVPLYKDPDDDLTLLILEEDRLLSGFVPLLAAPQDPCYVEKTSDKVIAADCKRVTVLKYFLEALCGQEEPLLAFKGGKYVSVAPVPDTMGKEMGSQEGTRLEDEEEDVVIEDFEEDSEAEGSGGEDDIRELRAKKLALARKIAEQQRRQEKIQAVLEDHSQMRQMELEIRPLFLVPDTNGFIDHLASLARLLESRKYILVVPLIVINELDGLAKGQETDHRAGGYARVVQEKARKSIEFLEQRFESRDSCLRALTSRGNELESIAFRSEDITGQLGNNDDLILSCCLHYCKDKAKDFMPASKEEPIRLLREVVLLTDDRNLRVKALTRNVPVRDIPAFLTWAQVG

SEQ ID NO: 13 - DNA, 3537 bp, Homo sapiens
atgagcctgcagagcgcgcagtacctccggcaggcagaagtcctgaaggctgacatgacagattctaagctgggtccagctgaagtctggacatccaggcaggctctgcaggacctgtaccagaaaatgctagttaccgatttggaatacgctttagacaagaaagtagaacaggatctctggaatcacgcctttaagaatcagatcacaacactacaaggccaggcaaagaatcgagcaaatccgaatcggagtgaagttcaggcaaacctttctctgttcctagaggcagctagtggcttctatactcagttattacaagaactgtgtacagtatttaatgtagatttaccatgccgtgtgaagtcttcccaattgggaattatcagcaataaacagacgcataccagcgccatagtgaagccacagtctagctcctgttcctatatctgccagcactgcctcgtccaccttggagacattgctcgatacagaaaccagaccagccaggcagagtcctactataggcatgcagctcagcttgtcccctccaatggtcagccttataatcagttggctatcttagcttcttccaaaggagaccatctgaccacaattttctactactgcagaagcattgctgtgaagttccctttcccagctgcctccactaatctgcaaaaagcactttctaaagcactggaaagccgagatgaggtgaaaaccaagtggggtgtttctgacttcatcaaggcctttattaaattccacggtcatgtgtacctgagtaagagcttggaaaagttgagccctcttcgagagaaattggaagaacagtttaagaggctgctattccaaaaagctttcaactctcagcagttagttcatgtcactgtcattaacctgtttcaacttcatcaccttcgtgactttagcaatgaaaccgagcagcacacttatagccaagatgagcagctatgttggacacagttgctggccctctttatgtcttttctcggcatcctgtgcaagtgtcctctacagaatgagtctcaggaggagtcctacaatgcctatcctcttccagcagtcaaggtctccatggactggctaagactcagacccagggtctttcaggaggcagtggtggatgaaagacagtacatttggccctggttgatttctcttctgaatagtttccatccccatgaagaggacctctcaagtattagtgcgacaccacttccagaggagtttgaattacaaggatttttggcattgagaccttctttcaggaacttggatttttccaaaggtcaccagggtattacaggggacaaagaaggccagcaacgacgaatacgacagcaacgcttgatctctataggcaaatggattgctgataatcagccaaggctgattcagtgtgaaaatgaggtagggaaattgttgtttatcacagaaatcccagaattaatactggaagaccccagtgaagccaaagagaacctcattctgcaagaaacatctgtgatagagtcgctggctgcagatgggagcccagggctaaaatcagtgctatctacaagccgaaatttaagcaacaactgtgacacaggagagaagccagtggttaccttcaaagaaaacattaagacacgagaagtgaacagagaccaaggaagaagttttcctcccaaagaggtaaaatcccagacagaactaagaaagactccagtgtctgaagccagaaaaacacctgtaactcaaaccccaactcaagcaagtaactcccagttcatccccattcatcaccctggagccttccctcctcttcccagcaggccagggtttccgcccccaacatatgttatccccccgcctgtggcattttctatgggctcaggttacaccttcccagctggtgtttctgtcccaggaacctttcttcagcctacagctcactctccagcaggaaaccaggtgcaagctgggaaacagtcccacattccttacagccagcaacggccctctggaccagggccaatgaaccagggacctcaacaatcacagccaccttcccagcaaccccttacatctttaccagctcagccaacagcacagtctacaagccagctgcaggttcaagctctaactcagcaacaacaatcccctacaaaagctgtgccggctttggggaaaagcccgcctcaccactctggattccagcagtatcaacaggcagatgcctccaaacagctgtggaatccccctcaggttcaaggcccattagggaaaattatgcctgtgaaacagccctactaccttcagacccaagaccccataaaactgtttgagccgtcattgcaacctcctgtaatgcagcagcagcctctagaaaaaaaaatgaagccttttcccatggagccatataaccataatccctcagaagtcaaggtcccagaattctactgggattcttcctacagcatggctgataacagatctgtaatggcacagcaagcaaacatagaccgcaggggcaaacggtcaccaggaatcttccgtccagagcaggatcctgtacccagaatgccgtttgaggaccccaagagctcccctctgcttcctccggacctgttaaagagtctggctgccttggaggaagaggaagagctgattttttctaacactcctgatctttacccggctctgctggggcctctcgcctctcttcctggacgaagcctttttaaatccttattggagaagccctcagagctcatgtcacattcatcctctttcctgtccctcaccggattctctctcaatcaggaaagatacccaaataatagtatgttcaatgaggtatatgggaaaaacctgacatccagctccaaagcagaactcagtccctcaatggccccccaggaaacatctctgtattccctttttgaagggactccgtggtctccatcacttcctgccagttcagatcattcaacaccagccagccagtctcctcattcctctaacccaagcagcctacccagctctcctccaacacacaaccataattctgttccattctccaattttggacccattgggactccagataacagggatagaaggactgcagatcggtggaaaactgataagccagccatgggtgggtttggcattgattatctctcagcaacgtcatcctctgagagcagttggcatcaggccagcactccgagtggcacctggacaggccatggcccttccatggaggattcctctgctgtcctcatggaaagcctaaagaagcaacagcatggggtccagcagttggggcccaaaagacagtctgaagaggaaggaagcagcagtatctgcgtagcccacagagggcccaggcccctgcccagctgcagtctcccagcctccactttcagagtgaaattcaaggcagcacggacatgtgcccatcaggcacagaagaaaacacgacgtcgtccattttggaagagacgaaagaaaggaaaataa

SEQ ID NO: 14 - protein, 1178 aa, Homo sapiens [sequence omitted]